European Patent Application EP 4 737 479 A1, published May 6, 2026. Title: 4-1BB结合蛋白. Applicant: 百奥泰生物制药股份有限公司. The sequence listing filed with the application follows.

SEQUENCE LISTING (42 sequences)

SEQ ID NO: 1 - protein, 128 aa, synthetic construct
EVQLVESGGGLVQPGGSLRLSCAASGFTFSSYAMGWVRQAPGKGREFVSAISGNGGSTYYADSVKGRFTISRDNSKNTLYLQMNSLRAEDTAVYYCAAGYSYLYPGGLSTRPSFYDYWGQGTQVTVSS

SEQ ID NO: 2 - protein, 128 aa, synthetic construct
EVQLVESGGGLVQPGGSLRLSCAASGFTFSSYAMGWVRQAPGKGREFVSAISGNGGSTYYADSVKGRFTISRDNSKNTLYLQMNSLRAEDTAVYYCAAGDAYVYPYGVSTDPSFYDYWGQGTQVTVSS

SEQ ID NO: 3 - protein, 128 aa, synthetic construct
EVQLVESGGGLVQPGGSLRLSCAASGFTFSSYAMGWVRQAPGKGREFVSAISGSGGSTYYADSVKGRFTISRDNSKNTLYLQMNSLRAEDTAVYYCAAGYSYLYPGGLSTRPSFYDYWGQGTQVTVSS

SEQ ID NO: 4 - protein, 128 aa, synthetic construct
EVQLVESGGGLVQPGGSLRLSCAASGFTFSSYAMGWVRQAPGKGREFVSAISGNGGSTFYADSVKGRFTISRDNSKNTLYLQMNSLRAEDTAVYYCAAGYSYLYPGGLSTRPSFYDYWGQGTQVTVSS

SEQ ID NO: 5 - protein, 128 aa, synthetic construct
EVQLVESGGGLVQPGGSLRLSCAASGFTFSSYAMGWVRQAPGKGREFVSAISGYGGTTYYADSVKGRFTISRDNSKNTLYLQMNSLRAEDTAVYYCAAGTGYYSRVGVSTDPSFYDYWGQGTQVTVSS

SEQ ID NO: 6 - protein, 128 aa, synthetic construct
EVQLVESGGGLVQPGGSLRLSCAASGFTFSSYAMGWVRQAPGKGREFVSAISGYGGSTYYADSVKGRFTISRDNSKNTLYLQMNSLRAEDTAVYYCAAGSGLYSSYGVSTDPSFYDYWGQGTQVTVSS

SEQ ID NO: 7 - protein, 5 aa, synthetic construct
SYAMG

SEQ ID NO: 8 - protein, 7 aa, synthetic construct
GNGGSTY

SEQ ID NO: 9 - protein, 7 aa, synthetic construct
GSGGSTY

SEQ ID NO: 10 - protein, 7 aa, synthetic construct
GNGGSTF

SEQ ID NO: 11 - protein, 7 aa, synthetic construct
GYGGTTY

SEQ ID NO: 12 - protein, 7 aa, synthetic construct
GSGGTTY

SEQ ID NO: 13 - protein, 7 aa, synthetic construct
GYGGSTY

SEQ ID NO: 14 - protein, 17 aa, synthetic construct
GYSYLYPGGLSTRPSFY

SEQ ID NO: 15 - protein, 17 aa, synthetic construct
GDAYVYPYGVSTDPSFY

SEQ ID NO: 16 - protein, 17 aa, synthetic construct
GTGYYSRVGVSTDPSFY

SEQ ID NO: 17 - protein, 17 aa, synthetic construct
GYSYLSPGGVSTRPSFY

SEQ ID NO: 18 - protein, 17 aa, synthetic construct
GSGLYSSYGVSTDPSFY

SEQ ID NO: 19 - protein, 17 aa, synthetic construct
GSAYGYSGGLSTDPSFY

SEQ ID NO: 20 - protein, 10 aa, synthetic construct
GGGGSGGGGS

SEQ ID NO: 21 - protein, 232 aa, synthetic construct
EPKSSDKTHTCPPCPAPELLGGPSVFLFPPKPKDTLMISRTPEVTCVVVDVSHEDPEVKFNWYVDGVEVHNAKTKPREEQYNSTYRVVSVLTVLHQDWLNGKEYKCKVSNKALPAPIEKTISKAKGQPREPQVYTLPPSRDELTKNQVSLTCLVKGFYPSDIAVEWESNGQPENNYKTTPPVLDSDGSFFLYSKLTVDKSRWQQGNVFSCSVMHEALHNHYTQKSLSLSPGK

SEQ ID NO: 22 - protein, 370 aa, synthetic construct
EVQLVESGGGLVQPGGSLRLSCAASGFTFSSYAMGWVRQAPGKGREFVSAISGNGGSTYYADSVKGRFTISRDNSKNTLYLQMNSLRAEDTAVYYCAAGYSYLYPGGLSTRPSFYDYWGQGTQVTVSSGGGGSGGGGSEPKSSDKTHTCPPCPAPELLGGPSVFLFPPKPKDTLMISRTPEVTCVVVDVSHEDPEVKFNWYVDGVEVHNAKTKPREEQYNSTYRVVSVLTVLHQDWLNGKEYKCKVSNKALPAPIEKTISKAKGQPREPQVYTLPPSRDELTKNQVSLTCLVKGFYPSDIAVEWESNGQPENNYKTTPPVLDSDGSFFLYSKLTVDKSRWQQGNVFSCSVMHEALHNHYTQKSLSLSPGK

SEQ ID NO: 23 - protein, 370 aa, synthetic construct
EVQLVESGGGLVQPGGSLRLSCAASGFTFSSYAMGWVRQAPGKGREFVSAISGNGGSTYYADSVKGRFTISRDNSKNTLYLQMNSLRAEDTAVYYCAAGDAYVYPYGVSTDPSFYDYWGQGTQVTVSSGGGGSGGGGSEPKSSDKTHTCPPCPAPELLGGPSVFLFPPKPKDTLMISRTPEVTCVVVDVSHEDPEVKFNWYVDGVEVHNAKTKPREEQYNSTYRVVSVLTVLHQDWLNGKEYKCKVSNKALPAPIEKTISKAKGQPREPQVYTLPPSRDELTKNQVSLTCLVKGFYPSDIAVEWESNGQPENNYKTTPPVLDSDGSFFLYSKLTVDKSRWQQGNVFSCSVMHEALHNHYTQKSLSLSPGK

SEQ ID NO: 24 - protein, 370 aa, synthetic construct
EVQLVESGGGLVQPGGSLRLSCAASGFTFSSYAMGWVRQAPGKGREFVSAISGSGGSTYYADSVKGRFTISRDNSKNTLYLQMNSLRAEDTAVYYCAAGYSYLYPGGLSTRPSFYDYWGQGTQVTVSSGGGGSGGGGSEPKSSDKTHTCPPCPAPELLGGPSVFLFPPKPKDTLMISRTPEVTCVVVDVSHEDPEVKFNWYVDGVEVHNAKTKPREEQYNSTYRVVSVLTVLHQDWLNGKEYKCKVSNKALPAPIEKTISKAKGQPREPQVYTLPPSRDELTKNQVSLTCLVKGFYPSDIAVEWESNGQPENNYKTTPPVLDSDGSFFLYSKLTVDKSRWQQGNVFSCSVMHEALHNHYTQKSLSLSPGK

SEQ ID NO: 25 - protein, 370 aa, synthetic construct
EVQLVESGGGLVQPGGSLRLSCAASGFTFSSYAMGWVRQAPGKGREFVSAISGNGGSTFYADSVKGRFTISRDNSKNTLYLQMNSLRAEDTAVYYCAAGYSYLYPGGLSTRPSFYDYWGQGTQVTVSSGGGGSGGGGSEPKSSDKTHTCPPCPAPELLGGPSVFLFPPKPKDTLMISRTPEVTCVVVDVSHEDPEVKFNWYVDGVEVHNAKTKPREEQYNSTYRVVSVLTVLHQDWLNGKEYKCKVSNKALPAPIEKTISKAKGQPREPQVYTLPPSRDELTKNQVSLTCLVKGFYPSDIAVEWESNGQPENNYKTTPPVLDSDGSFFLYSKLTVDKSRWQQGNVFSCSVMHEALHNHYTQKSLSLSPGK

SEQ ID NO: 26 - protein, 370 aa, synthetic construct
EVQLVESGGGLVQPGGSLRLSCAASGFTFSSYAMGWVRQAPGKGREFVSAISGYGGTTYYADSVKGRFTISRDNSKNTLYLQMNSLRAEDTAVYYCAAGTGYYSRVGVSTDPSFYDYWGQGTQVTVSSGGGGSGGGGSEPKSSDKTHTCPPCPAPELLGGPSVFLFPPKPKDTLMISRTPEVTCVVVDVSHEDPEVKFNWYVDGVEVHNAKTKPREEQYNSTYRVVSVLTVLHQDWLNGKEYKCKVSNKALPAPIEKTISKAKGQPREPQVYTLPPSRDELTKNQVSLTCLVKGFYPSDIAVEWESNGQPENNYKTTPPVLDSDGSFFLYSKLTVDKSRWQQGNVFSCSVMHEALHNHYTQKSLSLSPGK

SEQ ID NO: 27 - protein, 370 aa, synthetic construct
EVQLVESGGGLVQPGGSLRLSCAASGFTFSSYAMGWVRQAPGKGREFVSAISGYGGSTYYADSVKGRFTISRDNSKNTLYLQMNSLRAEDTAVYYCAAGSGLYSSYGVSTDPSFYDYWGQGTQVTVSSGGGGSGGGGSEPKSSDKTHTCPPCPAPELLGGPSVFLFPPKPKDTLMISRTPEVTCVVVDVSHEDPEVKFNWYVDGVEVHNAKTKPREEQYNSTYRVVSVLTVLHQDWLNGKEYKCKVSNKALPAPIEKTISKAKGQPREPQVYTLPPSRDELTKNQVSLTCLVKGFYPSDIAVEWESNGQPENNYKTTPPVLDSDGSFFLYSKLTVDKSRWQQGNVFSCSVMHEALHNHYTQKSLSLSPGK

SEQ ID NO: 28 - protein, 255 aa, synthetic construct
MGNSCYNIVATLLLVLNFERTRSLQDPCSNCPAGTFCDNNRNQICSPCPPNSFSSAGGQRTCDICRQCKGVFRTRKECSSTSNAECDCTPGFHCLGAGCSMCEQDCKQGQELTKKGCKDCCFGTFNDQKRGICRPWTNCSLDGKSVLVNGTKERDVVCGPSPADLSPGASSVTPPAPAREPGHSPQIISFFLALTSTALLFLLFFLTLRFSVVKRGRKKLLYIFKQPFMRPVQTTQEEDGCSCRFPEEEEGGCEL

SEQ ID NO: 29 - protein, 128 aa, synthetic construct
EVQLVESGGGLVQPGGSLRLSCAASGFTFSSYAMGWVRQAPGKGREFVSAISGNGGSTYYADSVKGRFTISRDNSKNTLYLQMNSLRAEDTAVYYCAAGYSYLSPGGVSTRPSFYDYWGQGTQVTVSS

SEQ ID NO: 30 - protein, 128 aa, synthetic construct
EVQLVESGGGLVQPGGSLRLSCAASGFTFSSYAMGWVRQAPGKGREFVSAISGSGGTTYYADSVKGRFTISRDNSKNTLYLQMNSLRAEDTAVYYCAAGTGYYSRVGVSTDPSFYDYWGQGTQVTVSS

SEQ ID NO: 31 - protein, 17 aa, synthetic construct
AISGNGGSTYYADSVKG

SEQ ID NO: 32 - protein, 17 aa, synthetic construct
AISGSGGSTYYADSVKG

SEQ ID NO: 33 - protein, 17 aa, synthetic construct
AISGNGGSTFYADSVKG

SEQ ID NO: 34 - protein, 17 aa, synthetic construct
AISGYGGTTYYADSVKG

SEQ ID NO: 35 - protein, 17 aa, synthetic construct
AISGSGGTTYYADSVKG

SEQ ID NO: 36 - protein, 17 aa, synthetic construct
AISGYGGSTYYADSVKG

SEQ ID NO: 37 - protein, 19 aa, synthetic construct
GYSYLYPGGLSTRPSFYDY

SEQ ID NO: 38 - protein, 19 aa, synthetic construct
GDAYVYPYGVSTDPSFYDY

SEQ ID NO: 39 - protein, 19 aa, synthetic construct
GTGYYSRVGVSTDPSFYDY

SEQ ID NO: 40 - protein, 19 aa, synthetic construct
GYSYLSPGGVSTRPSFYDY

SEQ ID NO: 41 - protein, 19 aa, synthetic construct
GSGLYSSYGVSTDPSFYDY

SEQ ID NO: 42 - protein, 19 aa, synthetic construct
GSAYGYSGGLSTDPSFYDY